European Patent Application EP 4 495 231 A1, published January 22, 2025. Title: Mature Polypeptide Sequence for Synthesizing Oligosachharide and Use. Applicant: Shandong Hengdu Biotech Co., Ltd. Application CN PCT/CN2023/109242, filed July 26, 2023. The sequence listing filed with the application follows.

SEQUENCE LISTING (25 sequences)

SEQ ID NO: 1 - protein, 747 aa, synthetic construct
  source 1..747: note = LNBP-M3
MTSTGRFTLPSEENFAEKTKELAELWGADAIRNSDGTHLDESVLALGKKIYSAYFPTRAHNEWITLHMDETPQVYLLTGRVLAEADIVDVPLMDGFFEEQLKPNRDADPHKYWEVVDRTTNEVVDASLWTLDEDTDTVHVSGATPMHEYTVSFLAYIIWDPVEMYNHLTNGWGDKEHEIPFDIYHPATRKFVFDTFEQWLKDNPQVDVVRFTTFFYQFTLLFDQKQREKVVDWFGCACTVSPAALDDFEKEYGYRLRPEDFVDGGAYNSAWRVPRKAQRDWIDFLSGFVRTNVKKLADMSHEAGKEAMMFLGDQWIGTEPYKDGFEDLGLDAVVGSIGDGTTTRMIADIPGVKYTEGRFLPYFFPDTFYEGNDPSIEGLDNWRKARRAILRSPISRMGYGGYLSLAAKFPKFVDTVTHIADEFRDIHDRTGGVAAEGELNVAILNSWGKMRSWMAFMGGNKQTYSYYGILESLSGMRVNVRFISFDDVLEHGVADDIDVIINGGPVDTAFTGGDVWKNPKLTETLRAWVRGGGAFVGVGEPSSLARFQAGRFFQLADVLGVDEERYQTLSVDKYFPAVTPEHFITADVHVDPAAREAWEKAGYRIPLSGCGGGQGIKPLGGIDFGEPIANTFPVNEDVTLLRADGGQVQLAVNEYGKGRGVYVSGLPYSAANARLLERALFWASHNEDKYTAYSSTNPECEVAVFPDAGQYCVINNTDRPQSTDVALPDGSVEHFDLDQSAIAWRNL

SEQ ID NO: 2 - protein, 747 aa, synthetic construct
  source 1..747: note = LNBP-M3-N460I
MTSTGRFTLPSEENFAEKTKELAELWGADAIRNSDGTHLDESVLALGKKIYSAYFPTRAHNEWITLHMDETPQVYLLTGRVLAEADIVDVPLMDGFFEEQLKPNRDADPHKYWEVVDRTTNEVVDASLWTLDEDTDTVHVSGATPMHEYTVSFLAYIIWDPVEMYNHLTNGWGDKEHEIPFDIYHPATRKFVFDTFEQWLKDNPQVDVVRFTTFFYQFTLLFDQKQREKVVDWFGCACTVSPAALDDFEKEYGYRLRPEDFVDGGAYNSAWRVPRKAQRDWIDFLSGFVRTNVKKLADMSHEAGKEAMMFLGDQWIGTEPYKDGFEDLGLDAVVGSIGDGTTTRMIADIPGVKYTEGRFLPYFFPDTFYEGNDPSIEGLDNWRKARRAILRSPISRMGYGGYLSLAAKFPKFVDTVTHIADEFRDIHDRTGGVAAEGELNVAILNSWGKMRSWMAFMGGIKQTYSYYGILESLSGMRVNVRFISFDDVLEHGVADDIDVIINGGPVDTAFTGGDVWKNPKLTETLRAWVRGGGAFVGVGEPSSLARFQAGRFFQLADVLGVDEERYQTLSVDKYFPAVTPEHFITADVHVDPAAREAWEKAGYRIPLSGCGGGQGIKPLGGIDFGEPIANTFPVNEDVTLLRADGGQVQLAVNEYGKGRGVYVSGLPYSAANARLLERALFWASHNEDKYTAYSSTNPECEVAVFPDAGQYCVINNTDRPQSTDVALPDGSVEHFDLDQSAIAWRNL

SEQ ID NO: 3 - protein, 747 aa, synthetic construct
  source 1..747: note = LNBP-M3-N460V
MTSTGRFTLPSEENFAEKTKELAELWGADAIRNSDGTHLDESVLALGKKIYSAYFPTRAHNEWITLHMDETPQVYLLTGRVLAEADIVDVPLMDGFFEEQLKPNRDADPHKYWEVVDRTTNEVVDASLWTLDEDTDTVHVSGATPMHEYTVSFLAYIIWDPVEMYNHLTNGWGDKEHEIPFDIYHPATRKFVFDTFEQWLKDNPQVDVVRFTTFFYQFTLLFDQKQREKVVDWFGCACTVSPAALDDFEKEYGYRLRPEDFVDGGAYNSAWRVPRKAQRDWIDFLSGFVRTNVKKLADMSHEAGKEAMMFLGDQWIGTEPYKDGFEDLGLDAVVGSIGDGTTTRMIADIPGVKYTEGRFLPYFFPDTFYEGNDPSIEGLDNWRKARRAILRSPISRMGYGGYLSLAAKFPKFVDTVTHIADEFRDIHDRTGGVAAEGELNVAILNSWGKMRSWMAFMGGVKQTYSYYGILESLSGMRVNVRFISFDDVLEHGVADDIDVIINGGPVDTAFTGGDVWKNPKLTETLRAWVRGGGAFVGVGEPSSLARFQAGRFFQLADVLGVDEERYQTLSVDKYFPAVTPEHFITADVHVDPAAREAWEKAGYRIPLSGCGGGQGIKPLGGIDFGEPIANTFPVNEDVTLLRADGGQVQLAVNEYGKGRGVYVSGLPYSAANARLLERALFWASHNEDKYTAYSSTNPECEVAVFPDAGQYCVINNTDRPQSTDVALPDGSVEHFDLDQSAIAWRNL

SEQ ID NO: 4 - protein, 747 aa, synthetic construct
  source 1..747: note = LNBP-M3-N460M
MTSTGRFTLPSEENFAEKTKELAELWGADAIRNSDGTHLDESVLALGKKIYSAYFPTRAHNEWITLHMDETPQVYLLTGRVLAEADIVDVPLMDGFFEEQLKPNRDADPHKYWEVVDRTTNEVVDASLWTLDEDTDTVHVSGATPMHEYTVSFLAYIIWDPVEMYNHLTNGWGDKEHEIPFDIYHPATRKFVFDTFEQWLKDNPQVDVVRFTTFFYQFTLLFDQKQREKVVDWFGCACTVSPAALDDFEKEYGYRLRPEDFVDGGAYNSAWRVPRKAQRDWIDFLSGFVRTNVKKLADMSHEAGKEAMMFLGDQWIGTEPYKDGFEDLGLDAVVGSIGDGTTTRMIADIPGVKYTEGRFLPYFFPDTFYEGNDPSIEGLDNWRKARRAILRSPISRMGYGGYLSLAAKFPKFVDTVTHIADEFRDIHDRTGGVAAEGELNVAILNSWGKMRSWMAFMGGMKQTYSYYGILESLSGMRVNVRFISFDDVLEHGVADDIDVIINGGPVDTAFTGGDVWKNPKLTETLRAWVRGGGAFVGVGEPSSLARFQAGRFFQLADVLGVDEERYQTLSVDKYFPAVTPEHFITADVHVDPAAREAWEKAGYRIPLSGCGGGQGIKPLGGIDFGEPIANTFPVNEDVTLLRADGGQVQLAVNEYGKGRGVYVSGLPYSAANARLLERALFWASHNEDKYTAYSSTNPECEVAVFPDAGQYCVINNTDRPQSTDVALPDGSVEHFDLDQSAIAWRNL

SEQ ID NO: 5 - protein, 747 aa, synthetic construct
  source 1..747: note = LNBP-M3-S608V
MTSTGRFTLPSEENFAEKTKELAELWGADAIRNSDGTHLDESVLALGKKIYSAYFPTRAHNEWITLHMDETPQVYLLTGRVLAEADIVDVPLMDGFFEEQLKPNRDADPHKYWEVVDRTTNEVVDASLWTLDEDTDTVHVSGATPMHEYTVSFLAYIIWDPVEMYNHLTNGWGDKEHEIPFDIYHPATRKFVFDTFEQWLKDNPQVDVVRFTTFFYQFTLLFDQKQREKVVDWFGCACTVSPAALDDFEKEYGYRLRPEDFVDGGAYNSAWRVPRKAQRDWIDFLSGFVRTNVKKLADMSHEAGKEAMMFLGDQWIGTEPYKDGFEDLGLDAVVGSIGDGTTTRMIADIPGVKYTEGRFLPYFFPDTFYEGNDPSIEGLDNWRKARRAILRSPISRMGYGGYLSLAAKFPKFVDTVTHIADEFRDIHDRTGGVAAEGELNVAILNSWGKMRSWMAFMGGNKQTYSYYGILESLSGMRVNVRFISFDDVLEHGVADDIDVIINGGPVDTAFTGGDVWKNPKLTETLRAWVRGGGAFVGVGEPSSLARFQAGRFFQLADVLGVDEERYQTLSVDKYFPAVTPEHFITADVHVDPAAREAWEKAGYRIPLVGCGGGQGIKPLGGIDFGEPIANTFPVNEDVTLLRADGGQVQLAVNEYGKGRGVYVSGLPYSAANARLLERALFWASHNEDKYTAYSSTNPECEVAVFPDAGQYCVINNTDRPQSTDVALPDGSVEHFDLDQSAIAWRNL

SEQ ID NO: 6 - protein, 747 aa, synthetic construct
  source 1..747: note = LNBP-M3-C236Y/D572V
MTSTGRFTLPSEENFAEKTKELAELWGADAIRNSDGTHLDESVLALGKKIYSAYFPTRAHNEWITLHMDETPQVYLLTGRVLAEADIVDVPLMDGFFEEQLKPNRDADPHKYWEVVDRTTNEVVDASLWTLDEDTDTVHVSGATPMHEYTVSFLAYIIWDPVEMYNHLTNGWGDKEHEIPFDIYHPATRKFVFDTFEQWLKDNPQVDVVRFTTFFYQFTLLFDQKQREKVVDWFGYACTVSPAALDDFEKEYGYRLRPEDFVDGGAYNSAWRVPRKAQRDWIDFLSGFVRTNVKKLADMSHEAGKEAMMFLGDQWIGTEPYKDGFEDLGLDAVVGSIGDGTTTRMIADIPGVKYTEGRFLPYFFPDTFYEGNDPSIEGLDNWRKARRAILRSPISRMGYGGYLSLAAKFPKFVDTVTHIADEFRDIHDRTGGVAAEGELNVAILNSWGKMRSWMAFMGGNKQTYSYYGILESLSGMRVNVRFISFDDVLEHGVADDIDVIINGGPVDTAFTGGDVWKNPKLTETLRAWVRGGGAFVGVGEPSSLARFQAGRFFQLADVLGVDEERYQTLSVVKYFPAVTPEHFITADVHVDPAAREAWEKAGYRIPLSGCGGGQGIKPLGGIDFGEPIANTFPVNEDVTLLRADGGQVQLAVNEYGKGRGVYVSGLPYSAANARLLERALFWASHNEDKYTAYSSTNPECEVAVFPDAGQYCVINNTDRPQSTDVALPDGSVEHFDLDQSAIAWRNL

SEQ ID NO: 7 - protein, 747 aa, synthetic construct
  source 1..747: note = LNBP-M3-C236Y/S608V
MTSTGRFTLPSEENFAEKTKELAELWGADAIRNSDGTHLDESVLALGKKIYSAYFPTRAHNEWITLHMDETPQVYLLTGRVLAEADIVDVPLMDGFFEEQLKPNRDADPHKYWEVVDRTTNEVVDASLWTLDEDTDTVHVSGATPMHEYTVSFLAYIIWDPVEMYNHLTNGWGDKEHEIPFDIYHPATRKFVFDTFEQWLKDNPQVDVVRFTTFFYQFTLLFDQKQREKVVDWFGYACTVSPAALDDFEKEYGYRLRPEDFVDGGAYNSAWRVPRKAQRDWIDFLSGFVRTNVKKLADMSHEAGKEAMMFLGDQWIGTEPYKDGFEDLGLDAVVGSIGDGTTTRMIADIPGVKYTEGRFLPYFFPDTFYEGNDPSIEGLDNWRKARRAILRSPISRMGYGGYLSLAAKFPKFVDTVTHIADEFRDIHDRTGGVAAEGELNVAILNSWGKMRSWMAFMGGNKQTYSYYGILESLSGMRVNVRFISFDDVLEHGVADDIDVIINGGPVDTAFTGGDVWKNPKLTETLRAWVRGGGAFVGVGEPSSLARFQAGRFFQLADVLGVDEERYQTLSVDKYFPAVTPEHFITADVHVDPAAREAWEKAGYRIPLVGCGGGQGIKPLGGIDFGEPIANTFPVNEDVTLLRADGGQVQLAVNEYGKGRGVYVSGLPYSAANARLLERALFWASHNEDKYTAYSSTNPECEVAVFPDAGQYCVINNTDRPQSTDVALPDGSVEHFDLDQSAIAWRNL

SEQ ID NO: 8 - protein, 747 aa, synthetic construct
  source 1..747: note = LNBP-M3-C236Y/N460M/S608V
MTSTGRFTLPSEENFAEKTKELAELWGADAIRNSDGTHLDESVLALGKKIYSAYFPTRAHNEWITLHMDETPQVYLLTGRVLAEADIVDVPLMDGFFEEQLKPNRDADPHKYWEVVDRTTNEVVDASLWTLDEDTDTVHVSGATPMHEYTVSFLAYIIWDPVEMYNHLTNGWGDKEHEIPFDIYHPATRKFVFDTFEQWLKDNPQVDVVRFTTFFYQFTLLFDQKQREKVVDWFGYACTVSPAALDDFEKEYGYRLRPEDFVDGGAYNSAWRVPRKAQRDWIDFLSGFVRTNVKKLADMSHEAGKEAMMFLGDQWIGTEPYKDGFEDLGLDAVVGSIGDGTTTRMIADIPGVKYTEGRFLPYFFPDTFYEGNDPSIEGLDNWRKARRAILRSPISRMGYGGYLSLAAKFPKFVDTVTHIADEFRDIHDRTGGVAAEGELNVAILNSWGKMRSWMAFMGGMKQTYSYYGILESLSGMRVNVRFISFDDVLEHGVADDIDVIINGGPVDTAFTGGDVWKNPKLTETLRAWVRGGGAFVGVGEPSSLARFQAGRFFQLADVLGVDEERYQTLSVDKYFPAVTPEHFITADVHVDPAAREAWEKAGYRIPLVGCGGGQGIKPLGGIDFGEPIANTFPVNEDVTLLRADGGQVQLAVNEYGKGRGVYVSGLPYSAANARLLERALFWASHNEDKYTAYSSTNPECEVAVFPDAGQYCVINNTDRPQSTDVALPDGSVEHFDLDQSAIAWRNL

SEQ ID NO: 9 - protein, 747 aa, synthetic construct
  source 1..747: note = LNBP-M3-C236Y
MTSTGRFTLPSEENFAEKTKELAELWGADAIRNSDGTHLDESVLALGKKIYSAYFPTRAHNEWITLHMDETPQVYLLTGRVLAEADIVDVPLMDGFFEEQLKPNRDADPHKYWEVVDRTTNEVVDASLWTLDEDTDTVHVSGATPMHEYTVSFLAYIIWDPVEMYNHLTNGWGDKEHEIPFDIYHPATRKFVFDTFEQWLKDNPQVDVVRFTTFFYQFTLLFDQKQREKVVDWFGYACTVSPAALDDFEKEYGYRLRPEDFVDGGAYNSAWRVPRKAQRDWIDFLSGFVRTNVKKLADMSHEAGKEAMMFLGDQWIGTEPYKDGFEDLGLDAVVGSIGDGTTTRMIADIPGVKYTEGRFLPYFFPDTFYEGNDPSIEGLDNWRKARRAILRSPISRMGYGGYLSLAAKFPKFVDTVTHIADEFRDIHDRTGGVAAEGELNVAILNSWGKMRSWMAFMGGNKQTYSYYGILESLSGMRVNVRFISFDDVLEHGVADDIDVIINGGPVDTAFTGGDVWKNPKLTETLRAWVRGGGAFVGVGEPSSLARFQAGRFFQLADVLGVDEERYQTLSVDKYFPAVTPEHFITADVHVDPAAREAWEKAGYRIPLSGCGGGQGIKPLGGIDFGEPIANTFPVNEDVTLLRADGGQVQLAVNEYGKGRGVYVSGLPYSAANARLLERALFWASHNEDKYTAYSSTNPECEVAVFPDAGQYCVINNTDRPQSTDVALPDGSVEHFDLDQSAIAWRNL

SEQ ID NO: 10 - protein, 747 aa, synthetic construct
  source 1..747: note = LNBP-M3-D572V
MTSTGRFTLPSEENFAEKTKELAELWGADAIRNSDGTHLDESVLALGKKIYSAYFPTRAHNEWITLHMDETPQVYLLTGRVLAEADIVDVPLMDGFFEEQLKPNRDADPHKYWEVVDRTTNEVVDASLWTLDEDTDTVHVSGATPMHEYTVSFLAYIIWDPVEMYNHLTNGWGDKEHEIPFDIYHPATRKFVFDTFEQWLKDNPQVDVVRFTTFFYQFTLLFDQKQREKVVDWFGCACTVSPAALDDFEKEYGYRLRPEDFVDGGAYNSAWRVPRKAQRDWIDFLSGFVRTNVKKLADMSHEAGKEAMMFLGDQWIGTEPYKDGFEDLGLDAVVGSIGDGTTTRMIADIPGVKYTEGRFLPYFFPDTFYEGNDPSIEGLDNWRKARRAILRSPISRMGYGGYLSLAAKFPKFVDTVTHIADEFRDIHDRTGGVAAEGELNVAILNSWGKMRSWMAFMGGNKQTYSYYGILESLSGMRVNVRFISFDDVLEHGVADDIDVIINGGPVDTAFTGGDVWKNPKLTETLRAWVRGGGAFVGVGEPSSLARFQAGRFFQLADVLGVDEERYQTLSVVKYFPAVTPEHFITADVHVDPAAREAWEKAGYRIPLSGCGGGQGIKPLGGIDFGEPIANTFPVNEDVTLLRADGGQVQLAVNEYGKGRGVYVSGLPYSAANARLLERALFWASHNEDKYTAYSSTNPECEVAVFPDAGQYCVINNTDRPQSTDVALPDGSVEHFDLDQSAIAWRNL

SEQ ID NO: 11 - DNA, 40 bp, synthetic construct
  source 1..40: mol_type = other DNA
atgggtggaaacaagcagacgtattcgtattacggcattc

SEQ ID NO: 12 - DNA, 27 bp, synthetic construct
  source 1..27: mol_type = other DNA
gaacgccatccacgaacgcatcttgcc

SEQ ID NO: 13 - DNA, 33 bp, synthetic construct
  source 1..33: mol_type = other DNA
ttcggctacgcctgcaccgtgagcccggccgcg

SEQ ID NO: 14 - DNA, 39 bp, synthetic construct
  source 1..39: mol_type = other DNA
gcaggcgtagccgaaccagtccacgaccttctcgcgctg

SEQ ID NO: 15 - DNA, 36 bp, synthetic construct
  source 1..36: mol_type = other DNA
gggtggaatcaagcagacgtattcgtattacggcat

SEQ ID NO: 16 - DNA, 32 bp, synthetic construct
  source 1..32: mol_type = other DNA
ctgcttgattccacccatgaacgccatccacg

SEQ ID NO: 17 - DNA, 36 bp, synthetic construct
  source 1..36: mol_type = other DNA
gggtggagtcaagcagacgtattcgtattacggcat

SEQ ID NO: 18 - DNA, 32 bp, synthetic construct
  source 1..32: mol_type = other DNA
ctgcttgactccacccatgaacgccatccacg

SEQ ID NO: 19 - DNA, 36 bp, synthetic construct
  source 1..36: mol_type = other DNA
gggtggaatgaagcagacgtattcgtattacggcat

SEQ ID NO: 20 - DNA, 32 bp, synthetic construct
  source 1..32: mol_type = other DNA
ctgcttcattccacccatgaacgccatccacg

SEQ ID NO: 21 - DNA, 34 bp, synthetic construct
  source 1..34: mol_type = other DNA
gtcggtggtcaagtacttcccggccgtcacgccg

SEQ ID NO: 22 - DNA, 39 bp, synthetic construct
  source 1..39: mol_type = other DNA
gtacttgaccaccgacagcgtctggtagcgttcctcgtc

SEQ ID NO: 23 - DNA, 33 bp, synthetic construct
  source 1..33: mol_type = other DNA
ccgctggtgggctgcggcggtggccagggcatc

SEQ ID NO: 24 - DNA, 41 bp, synthetic construct
  source 1..41: mol_type = other DNA
gcagcccaccagcgggatgcggtatccggccttctcccacg

SEQ ID NO: 25 - DNA, 2244 bp, synthetic construct
  source 1..2244: mol_type = other DNA; note = LNBP-M3
atgaccagcactggccgcttcacattgcccagtgaagagaacttcgctgaaaaaaccaaggaacttgctgaattgtggggcgctgatgccatccgtaattccgatggcacacaccttgacgagtccgtgctcgcactcggcaagaagatctacagcgcctactttccgacccgtgcacacaacgagtggatcacgctgcacatggacgagaccccgcaggtgtacttgctcaccgggcgcgtcctggcggaagcggacatcgtggatgttcccctgatggacggcttcttcgaggagcagctcaagccgaaccgtgacgccgacccgcacaagtactgggaagtcgtggaccgcaccaccaatgaggtcgtggatgcctccctgtggacgcttgatgaggacaccgataccgtgcatgtctccggcgcgacgccgatgcacgagtacacggtctcgttcctcgcgtacatcatctgggatccggtcgagatgtacaaccacctgacgaacgggtggggcgacaaggagcacgagattccgttcgatatctaccacccggcgacacgcaagttcgtgttcgacacgttcgagcagtggctcaaggacaacccgcaggtggatgtcgtgcgtttcacgacgttcttctaccagttcacgctgctgttcgaccagaagcagcgcgagaaggtcgtggactggttcggctgcgcctgcaccgtgagcccggccgcgctcgacgacttcgagaaggagtacggctaccgcctgcgccccgaagacttcgtagatggcggcgcctataactctgcgtggcgcgtgccgcgcaaggcccaacgcgactggatcgacttcctctccggtttcgttcgcaccaatgtcaagaagctcgccgacatgtcgcacgaggccggcaaggaagcgatgatgttcctgggtgaccagtggatcggtaccgagccgtacaaggatggtttcgaggatctgggcctggatgctgtcgtcggttcgatcggtgacggcaccacgacccgcatgatcgcggacatcccgggcgtgaagtacacggagggtcgtttcctgccgtacttcttccccgacacgttctacgagggcaacgacccgagcatcgaaggtctcgacaactggcgtaaagcgcgtcgtgccatcctgcgttccccgatttcgcgtatgggctacggcggatacctgtcgctggccgcgaagttcccgaagttcgtcgataccgtcacccacatcgccgacgagttccgcgacatccatgaccgtaccggtggagtcgccgccgaaggcgagctcaacgtggcgattctgaactcgtggggcaagatgcgttcgtggatggcgttcatgggtggaaacaagcagacgtattcgtattacggcattctggagtcgctgtcgggcatgcgcgtgaacgtgcggttcatcagcttcgatgacgtgctggagcatggcgtcgccgacgacatcgacgtgatcatcaacggtggcccggtcgacaccgcgttcaccggtggagacgtgtggaagaacccgaagctgaccgagaccctgcgtgcctgggtgcgcggcggcggagcattcgtcggcgttggagagcccagttcgctggcccgtttccaggctggtcgtttcttccagctggccgacgtgctgggcgtggacgaggaacgctaccagacgctgtcggtggacaagtacttcccggccgtcacgccggagcacttcatcaccgccgacgtgcatgtcgatcccgccgcccgcgaagcgtgggagaaggccggataccgcatcccgctgtcgggctgcggcggtggccagggcatcaaaccgcttggcggcatcgacttcggcgagccgatcgcgaacacgttcccggtcaacgaggacgtgacgctgctgcgtgccgacggcggtcaggtgcagctcgcggtcaacgagtacggcaagggccgcggcgtatacgtctccggtctgccctattcggccgcgaacgcccgtctgctggagcgtgccctgttctgggcctcccacaacgaggacaagtacacggcatacagctccaccaaccccgagtgcgaggtcgcggtgttccccgatgccggccagtactgcgtgatcaacaacaccgaccgtccgcagtccacggatgtggctctgcctgacggttcggtcgagcatttcgacctcgaccagagcgccatcgcttggcgcaacctctga